European Patent Application EP 4 130 032 A1, published February 8, 2023. Title: Reagent containing antibody having partial deletion of FC region. Applicant: Denka Company Limited. Application EP21774329.3. The sequence listing filed with the application follows.

SEQUENCE LISTING (36 sequences)

SEQ ID NO: 1 - protein, 218 aa, Mus musculus
DIVLTQSPGSLTVSLGQRATISCRASESVDNFGKSFMHWYQQKPGQSPKLLIYRASNREFGIPARFNGSGSGTDFALTINPVEADDVATYFCQQSNEDPRTFGGGTKLEIKRADAAPTVSIFPPSSEQLTSGGASVVCFLNNFYPKDINVKWKIDGSERQNGVLNSWTDQDSKDSTYSMSSTLTLTKDEYERHNSYTCEATHKTSTSPIVKSFNRNEC

SEQ ID NO: 2 - protein, 444 aa, Mus musculus
EVHLQQSGPELVKPGASVKMSCKTSGYTFTEYTIHWMKQSHGKSLEWIGGIFPNNGDTTYNQKFKVRATLTVGRSSSTAYMDLRSLTSEDSAVYYCVRNYGSSYGYFDVWGAGTTVTVSSAKTTPPSVYPLAPGSAAQTNSMVTLGCLVKGYFPEPVTVTWNSGSLSSGVHTFPAVLQSDLYTLSSSVTVPSSTWPSETVTCNVAHPASSTKVDKKIVPRDCGCKPCICTVPEVSSVFIFPPKPKDVLTITLTPKVTCVVVDISKDDPEVQFSWFVDDVEVHTAQTQPREEQFNSTFRSVSELPIMHQDWLNGKEFKCRVNSAAFPAPIEKTISKTKGRPKAPQVYTIPPPKEQMAKDKVSLTCMITDFFPEDITVEWQWNGQPAENYKNTQPIMDTDGSYFVYSKLNVQKSNWEAGNTFTCSVLHEGLHNHHTEKSLSHSPGK

SEQ ID NO: 3 - protein, 214 aa, Mus musculus
DILLTQSPAILSVSPGERVRLSCRASQSCGTSIYWYQQRTNGSPRLLIMYASEPFSGIPSRFSGSGSGTDFTLSINSVESEDIADYYCQQSNSWPWTFGGGTRLEIKRADAAPTVSIFPPSSEQLTSGGASVVCFLNNFYPKDINVKWKIDGSERQNGVLNSWTDQDSKDSTYSMSSTLTLTKDEYERHNSYTCEATHKTSTSPIVKSFNRNEC

SEQ ID NO: 4 - protein, 438 aa, Mus musculus
QVQLQQSGAELARPGASVKLSCKASGYTFTSQWLQWVKQRPGQGLEWIGAIYPGDGDTRYTQKFKGKATLTADKSSSTAYMQLTNLAPEDSAVYYCARSSMDYWGQGTSVTVSSAKTTPPSVYPLAPGSAAQTNSMVTLGCLVKGYFPEPVTVTWNSGSLSSGVHTFPAVLQSDLYTLSSSVTVPSSTWPSETVTCNVAHPASSTKVDKKIVPRDCGCKPCICTVPEVSSVFIFPPKPKDVLTITLTPKVTCVVVDISKDDPEVQFSWFVDDVEVHTAQTQPREEQFNSTFRSVSELPIMHQDWLNGKEFKCRVNSAAFPAPIEKTISKTKGRPKAPQVYTIPPPKEQMAKDKVSLTCMITDFFPEDITVEWQWNGQPAENYKNTQPIMDTDGSYFVYSKLNVQKSNWEAGNTFTCSVLHEGLHNHHTEKSLSHSPGK

SEQ ID NO: 5 - protein, 348 aa, Artificial Sequence
  Delta 341-447
EVHLQQSGPELVKPGASVKMSCKTSGYTFTEYTIHWMKQSHGKSLEWIGGIFPNNGDTTYNQKFKVRATLTVGRSSSTAYMDLRSLTSEDSAVYYCVRNYGSSYGYFDVWGAGTTVTVSSAKTTPPSVYPLAPGSAAQTNSMVTLGCLVKGYFPEPVTVTWNSGSLSSGVHTFPAVLQSDLYTLSSSVTVPSSTWPSETVTCNVAHPASSTKVDKKIVPRDCGCKPCICTVPEVSSVFIFPPKPKDVLTITLTPKVTCVVVDISKDDPEVQFSWFVDDVEVHTAQTQPREEQFNSTFRSVSELPIMHQDWLNGKEFKCRVNSAAFPAPIEKTISKTKGGGGSHHHHHH

SEQ ID NO: 6 - protein, 342 aa, Artificial Sequence
  delta 341-447
QVQLQQSGAELARPGASVKLSCKASGYTFTSQWLQWVKQRPGQGLEWIGAIYPGDGDTRYTQKFKGKATLTADKSSSTAYMQLTNLAPEDSAVYYCARSSMDYWGQGTSVTVSSAKTTPPSVYPLAPGSAAQTNSMVTLGCLVKGYFPEPVTVTWNSGSLSSGVHTFPAVLQSDLYTLSSSVTVPSSTWPSETVTCNVAHPASSTKVDKKIVPRDCGCKPCICTVPEVSSVFIFPPKPKDVLTITLTPKVTCVVVDISKDDPEVQFSWFVDDVEVHTAQTQPREEQFNSTFRSVSELPIMHQDWLNGKEFKCRVNSAAFPAPIEKTISKTKGGGGSHHHHHH

SEQ ID NO: 7 - protein, 338 aa, Artificial Sequence
  delta 331-447
EVHLQQSGPELVKPGASVKMSCKTSGYTFTEYTIHWMKQSHGKSLEWIGGIFPNNGDTTYNQKFKVRATLTVGRSSSTAYMDLRSLTSEDSAVYYCVRNYGSSYGYFDVWGAGTTVTVSSAKTTPPSVYPLAPGSAAQTNSMVTLGCLVKGYFPEPVTVTWNSGSLSSGVHTFPAVLQSDLYTLSSSVTVPSSTWPSETVTCNVAHPASSTKVDKKIVPRDCGCKPCICTVPEVSSVFIFPPKPKDVLTITLTPKVTCVVVDISKDDPEVQFSWFVDDVEVHTAQTQPREEQFNSTFRSVSELPIMHQDWLNGKEFKCRVNSAAFPAGGGGSHHHHHH

SEQ ID NO: 8 - protein, 332 aa, Artificial Sequence
  delta 331-447
QVQLQQSGAELARPGASVKLSCKASGYTFTSQWLQWVKQRPGQGLEWIGAIYPGDGDTRYTQKFKGKATLTADKSSSTAYMQLTNLAPEDSAVYYCARSSMDYWGQGTSVTVSSAKTTPPSVYPLAPGSAAQTNSMVTLGCLVKGYFPEPVTVTWNSGSLSSGVHTFPAVLQSDLYTLSSSVTVPSSTWPSETVTCNVAHPASSTKVDKKIVPRDCGCKPCICTVPEVSSVFIFPPKPKDVLTITLTPKVTCVVVDISKDDPEVQFSWFVDDVEVHTAQTQPREEQFNSTFRSVSELPIMHQDWLNGKEFKCRVNSAAFPAGGGGSHHHHHH

SEQ ID NO: 9 - protein, 343 aa, Artificial Sequence
  delta 336-447
EVHLQQSGPELVKPGASVKMSCKTSGYTFTEYTIHWMKQSHGKSLEWIGGIFPNNGDTTYNQKFKVRATLTVGRSSSTAYMDLRSLTSEDSAVYYCVRNYGSSYGYFDVWGAGTTVTVSSAKTTPPSVYPLAPGSAAQTNSMVTLGCLVKGYFPEPVTVTWNSGSLSSGVHTFPAVLQSDLYTLSSSVTVPSSTWPSETVTCNVAHPASSTKVDKKIVPRDCGCKPCICTVPEVSSVFIFPPKPKDVLTITLTPKVTCVVVDISKDDPEVQFSWFVDDVEVHTAQTQPREEQFNSTFRSVSELPIMHQDWLNGKEFKCRVNSAAFPAPIEKTGGGGSHHHHHH

SEQ ID NO: 10 - protein, 337 aa, Artificial Sequence
  delta 336-447
QVQLQQSGAELARPGASVKLSCKASGYTFTSQWLQWVKQRPGQGLEWIGAIYPGDGDTRYTQKFKGKATLTADKSSSTAYMQLTNLAPEDSAVYYCARSSMDYWGQGTSVTVSSAKTTPPSVYPLAPGSAAQTNSMVTLGCLVKGYFPEPVTVTWNSGSLSSGVHTFPAVLQSDLYTLSSSVTVPSSTWPSETVTCNVAHPASSTKVDKKIVPRDCGCKPCICTVPEVSSVFIFPPKPKDVLTITLTPKVTCVVVDISKDDPEVQFSWFVDDVEVHTAQTQPREEQFNSTFRSVSELPIMHQDWLNGKEFKCRVNSAAFPAPIEKTGGGGSHHHHHH

SEQ ID NO: 11 - protein, 353 aa, Artificial Sequence
  delta 346-447
EVHLQQSGPELVKPGASVKMSCKTSGYTFTEYTIHWMKQSHGKSLEWIGGIFPNNGDTTYNQKFKVRATLTVGRSSSTAYMDLRSLTSEDSAVYYCVRNYGSSYGYFDVWGAGTTVTVSSAKTTPPSVYPLAPGSAAQTNSMVTLGCLVKGYFPEPVTVTWNSGSLSSGVHTFPAVLQSDLYTLSSSVTVPSSTWPSETVTCNVAHPASSTKVDKKIVPRDCGCKPCICTVPEVSSVFIFPPKPKDVLTITLTPKVTCVVVDISKDDPEVQFSWFVDDVEVHTAQTQPREEQFNSTFRSVSELPIMHQDWLNGKEFKCRVNSAAFPAPIEKTISKTKGRPKAGGGGSHHHHHH

SEQ ID NO: 12 - protein, 347 aa, Artificial Sequence
  delta 346-447
QVQLQQSGAELARPGASVKLSCKASGYTFTSQWLQWVKQRPGQGLEWIGAIYPGDGDTRYTQKFKGKATLTADKSSSTAYMQLTNLAPEDSAVYYCARSSMDYWGQGTSVTVSSAKTTPPSVYPLAPGSAAQTNSMVTLGCLVKGYFPEPVTVTWNSGSLSSGVHTFPAVLQSDLYTLSSSVTVPSSTWPSETVTCNVAHPASSTKVDKKIVPRDCGCKPCICTVPEVSSVFIFPPKPKDVLTITLTPKVTCVVVDISKDDPEVQFSWFVDDVEVHTAQTQPREEQFNSTFRSVSELPIMHQDWLNGKEFKCRVNSAAFPAPIEKTISKTKGRPKAGGGGSHHHHHH

SEQ ID NO: 13 - protein, 358 aa, Artificial Sequence
  delta 351-447
EVHLQQSGPELVKPGASVKMSCKTSGYTFTEYTIHWMKQSHGKSLEWIGGIFPNNGDTTYNQKFKVRATLTVGRSSSTAYMDLRSLTSEDSAVYYCVRNYGSSYGYFDVWGAGTTVTVSSAKTTPPSVYPLAPGSAAQTNSMVTLGCLVKGYFPEPVTVTWNSGSLSSGVHTFPAVLQSDLYTLSSSVTVPSSTWPSETVTCNVAHPASSTKVDKKIVPRDCGCKPCICTVPEVSSVFIFPPKPKDVLTITLTPKVTCVVVDISKDDPEVQFSWFVDDVEVHTAQTQPREEQFNSTFRSVSELPIMHQDWLNGKEFKCRVNSAAFPAPIEKTISKTKGRPKAPQVYTGGGGSHHHHHH

SEQ ID NO: 14 - protein, 291 aa, Artificial Sequence
  delta 351-447
QVQLQQSGAELARPGASVKLSCKASGYTFTSQWLQWVKQRPGQGLEWIGAIYPGDGDTRYTQKFKGKATLTADKSSSTAYMQLTNLAPEDSAVYYCARSSMDYWGQGTSVTVSSAKTTPPSVYPLAPGSAAQTNSMVTLGCLVKGYFPEPVTVTWNSGSLSSGVHTFPAVLQSDLYTLSSSVTVPSSTWPSETVTCNVAHPASSTKVDKKIVPRDCGCKPCICTVPEVSSVFIFPPKPKDVLTITLTPKVTCVVVDISKDDPEVQFSWFVDDVEVHTAQTQPREEQFNSTF

SEQ ID NO: 15 - protein, 5 aa, Artificial Sequence
  GS linker
GGGGS

SEQ ID NO: 16 - protein, 10 aa, Artificial Sequence
  GS linker
GGGGSGGGGS

SEQ ID NO: 17 - protein, 15 aa, Artificial Sequence
  GS linker
GGGGSGGGGSGGGGS

SEQ ID NO: 18 - protein, 20 aa, Artificial Sequence
  GS linker
GGGGSGGGGSGGGGSGGGGS

SEQ ID NO: 19 - protein, 348 aa, Artificial Sequence
  delta 231-340
EVHLQQSGPELVKPGASVKMSCKTSGYTFTEYTIHWMKQSHGKSLEWIGGIFPNNGDTTYNQKFKVRATLTVGRSSSTAYMDLRSLTSEDSAVYYCVRNYGSSYGYFDVWGAGTTVTVSSAKTTPPSVYPLAPGSAAQTNSMVTLGCLVKGYFPEPVTVTWNSGSLSSGVHTFPAVLQSDLYTLSSSVTVPSSTWPSETVTCNVAHPASSTKVDKKIVPRDCGCKPCICTGRPKAPQVYTIPPPKEQMAKDKVSLTCMITDFFPEDITVEWQWNGQPAENYKNTQPIMDTDGSYFVYSKLNVQKSNWEAGNTFTCSVLHEGLHNHHTEKSLSHSPGKGGGGSHHHHHH

SEQ ID NO: 20 - protein, 342 aa, Artificial Sequence
  delta 231-340
QVQLQQSGAELARPGASVKLSCKASGYTFTSQWLQWVKQRPGQGLEWIGAIYPGDGDTRYTQKFKGKATLTADKSSSTAYMQLTNLAPEDSAVYYCARSSMDYWGQGTSVTVSSAKTTPPSVYPLAPGSAAQTNSMVTLGCLVKGYFPEPVTVTWNSGSLSSGVHTFPAVLQSDLYTLSSSVTVPSSTWPSETVTCNVAHPASSTKVDKKIVPRDCGCKPCICTGRPKAPQVYTIPPPKEQMAKDKVSLTCMITDFFPEDITVEWQWNGQPAENYKNTQPIMDTDGSYFVYSKLNVQKSNWEAGNTFTCSVLHEGLHNHHTEKSLSHSPGKGGGGSHHHHHH

SEQ ID NO: 21 - protein, 353 aa, Artificial Sequence
  delta 231-340
EVHLQQSGPELVKPGASVKMSCKTSGYTFTEYTIHWMKQSHGKSLEWIGGIFPNNGDTTYNQKFKVRATLTVGRSSSTAYMDLRSLTSEDSAVYYCVRNYGSSYGYFDVWGAGTTVTVSSAKTTPPSVYPLAPGSAAQTNSMVTLGCLVKGYFPEPVTVTWNSGSLSSGVHTFPAVLQSDLYTLSSSVTVPSSTWPSETVTCNVAHPASSTKVDKKIVPRDCGCKPCICTGGGGSGRPKAPQVYTIPPPKEQMAKDKVSLTCMITDFFPEDITVEWQWNGQPAENYKNTQPIMDTDGSYFVYSKLNVQKSNWEAGNTFTCSVLHEGLHNHHTEKSLSHSPGKGGGGSHHHHHH

SEQ ID NO: 22 - protein, 347 aa, Artificial Sequence
  delta 231-340
QVQLQQSGAELARPGASVKLSCKASGYTFTSQWLQWVKQRPGQGLEWIGAIYPGDGDTRYTQKFKGKATLTADKSSSTAYMQLTNLAPEDSAVYYCARSSMDYWGQGTSVTVSSAKTTPPSVYPLAPGSAAQTNSMVTLGCLVKGYFPEPVTVTWNSGSLSSGVHTFPAVLQSDLYTLSSSVTVPSSTWPSETVTCNVAHPASSTKVDKKIVPRDCGCKPCICTGGGGSGRPKAPQVYTIPPPKEQMAKDKVSLTCMITDFFPEDITVEWQWNGQPAENYKNTQPIMDTDGSYFVYSKLNVQKSNWEAGNTFTCSVLHEGLHNHHTEKSLSHSPGKGGGGSHHHHHH

SEQ ID NO: 23 - protein, 358 aa, Artificial Sequence
  delta 231-340
EVHLQQSGPELVKPGASVKMSCKTSGYTFTEYTIHWMKQSHGKSLEWIGGIFPNNGDTTYNQKFKVRATLTVGRSSSTAYMDLRSLTSEDSAVYYCVRNYGSSYGYFDVWGAGTTVTVSSAKTTPPSVYPLAPGSAAQTNSMVTLGCLVKGYFPEPVTVTWNSGSLSSGVHTFPAVLQSDLYTLSSSVTVPSSTWPSETVTCNVAHPASSTKVDKKIVPRDCGCKPCICTGGGGSGGGGSGRPKAPQVYTIPPPKEQMAKDKVSLTCMITDFFPEDITVEWQWNGQPAENYKNTQPIMDTDGSYFVYSKLNVQKSNWEAGNTFTCSVLHEGLHNHHTEKSLSHSPGKGGGGSHHHHHH

SEQ ID NO: 24 - protein, 352 aa, Artificial Sequence
  delta 231-340
QVQLQQSGAELARPGASVKLSCKASGYTFTSQWLQWVKQRPGQGLEWIGAIYPGDGDTRYTQKFKGKATLTADKSSSTAYMQLTNLAPEDSAVYYCARSSMDYWGQGTSVTVSSAKTTPPSVYPLAPGSAAQTNSMVTLGCLVKGYFPEPVTVTWNSGSLSSGVHTFPAVLQSDLYTLSSSVTVPSSTWPSETVTCNVAHPASSTKVDKKIVPRDCGCKPCICTGGGGSGGGGSGRPKAPQVYTIPPPKEQMAKDKVSLTCMITDFFPEDITVEWQWNGQPAENYKNTQPIMDTDGSYFVYSKLNVQKSNWEAGNTFTCSVLHEGLHNHHTEKSLSHSPGKGGGGSHHHHHH

SEQ ID NO: 25 - protein, 363 aa, Artificial Sequence
  delta 231-340
EVHLQQSGPELVKPGASVKMSCKTSGYTFTEYTIHWMKQSHGKSLEWIGGIFPNNGDTTYNQKFKVRATLTVGRSSSTAYMDLRSLTSEDSAVYYCVRNYGSSYGYFDVWGAGTTVTVSSAKTTPPSVYPLAPGSAAQTNSMVTLGCLVKGYFPEPVTVTWNSGSLSSGVHTFPAVLQSDLYTLSSSVTVPSSTWPSETVTCNVAHPASSTKVDKKIVPRDCGCKPCICTGGGGSGGGGSGGGGSGRPKAPQVYTIPPPKEQMAKDKVSLTCMITDFFPEDITVEWQWNGQPAENYKNTQPIMDTDGSYFVYSKLNVQKSNWEAGNTFTCSVLHEGLHNHHTEKSLSHSPGKGGGGSHHHHHH

SEQ ID NO: 26 - protein, 357 aa, Artificial Sequence
  delta 231-340
QVQLQQSGAELARPGASVKLSCKASGYTFTSQWLQWVKQRPGQGLEWIGAIYPGDGDTRYTQKFKGKATLTADKSSSTAYMQLTNLAPEDSAVYYCARSSMDYWGQGTSVTVSSAKTTPPSVYPLAPGSAAQTNSMVTLGCLVKGYFPEPVTVTWNSGSLSSGVHTFPAVLQSDLYTLSSSVTVPSSTWPSETVTCNVAHPASSTKVDKKIVPRDCGCKPCICTGGGGSGGGGSGGGGSGRPKAPQVYTIPPPKEQMAKDKVSLTCMITDFFPEDITVEWQWNGQPAENYKNTQPIMDTDGSYFVYSKLNVQKSNWEAGNTFTCSVLHEGLHNHHTEKSLSHSPGKGGGGSHHHHHH

SEQ ID NO: 27 - protein, 368 aa, Artificial Sequence
  delta 231-340
EVHLQQSGPELVKPGASVKMSCKTSGYTFTEYTIHWMKQSHGKSLEWIGGIFPNNGDTTYNQKFKVRATLTVGRSSSTAYMDLRSLTSEDSAVYYCVRNYGSSYGYFDVWGAGTTVTVSSAKTTPPSVYPLAPGSAAQTNSMVTLGCLVKGYFPEPVTVTWNSGSLSSGVHTFPAVLQSDLYTLSSSVTVPSSTWPSETVTCNVAHPASSTKVDKKIVPRDCGCKPCICTGGGGSGGGGSGGGGSGGGGSGRPKAPQVYTIPPPKEQMAKDKVSLTCMITDFFPEDITVEWQWNGQPAENYKNTQPIMDTDGSYFVYSKLNVQKSNWEAGNTFTCSVLHEGLHNHHTEKSLSHSPGKGGGGSHHHHHH

SEQ ID NO: 28 - protein, 362 aa, Artificial Sequence
  delta 231-340
QVQLQQSGAELARPGASVKLSCKASGYTFTSQWLQWVKQRPGQGLEWIGAIYPGDGDTRYTQKFKGKATLTADKSSSTAYMQLTNLAPEDSAVYYCARSSMDYWGQGTSVTVSSAKTTPPSVYPLAPGSAAQTNSMVTLGCLVKGYFPEPVTVTWNSGSLSSGVHTFPAVLQSDLYTLSSSVTVPSSTWPSETVTCNVAHPASSTKVDKKIVPRDCGCKPCICTGGGGSGGGGSGGGGSGGGGSGRPKAPQVYTIPPPKEQMAKDKVSLTCMITDFFPEDITVEWQWNGQPAENYKNTQPIMDTDGSYFVYSKLNVQKSNWEAGNTFTCSVLHEGLHNHHTEKSLSHSPGKGGGGSHHHHHH

SEQ ID NO: 29 - protein, 367 aa, Artificial Sequence
  delta 231-330
EVHLQQSGPELVKPGASVKMSCKTSGYTFTEYTIHWMKQSHGKSLEWIGGIFPNNGDTTYNQKFKVRATLTVGRSSSTAYMDLRSLTSEDSAVYYCVRNYGSSYGYFDVWGAGTTVTVSSAKTTPPSVYPLAPGSAAQTNSMVTLGCLVKGYFPEPVTVTWNSGSLSSGVHTFPAVLQSDLYTLSSSVTVPSSTWPSETVTCNVAHPASSTKVDKKIVPRDCGCKPCICTGGGGSGGGGSGGGGSGGGGSPIEKTISKTKGRPKAPQVYTIPPPKEQMAKDKVSLTCMITDFFPEDITVEWQWNGQPAENYKNTQPIMDTDGSYFVYSKLNVQKSNWEAGNTFTCSVLHEGLHNHHTEKSLSHSPGK

SEQ ID NO: 30 - protein, 361 aa, Artificial Sequence
  delta 231-330
QVQLQQSGAELARPGASVKLSCKASGYTFTSQWLQWVKQRPGQGLEWIGAIYPGDGDTRYTQKFKGKATLTADKSSSTAYMQLTNLAPEDSAVYYCARSSMDYWGQGTSVTVSSAKTTPPSVYPLAPGSAAQTNSMVTLGCLVKGYFPEPVTVTWNSGSLSSGVHTFPAVLQSDLYTLSSSVTVPSSTWPSETVTCNVAHPASSTKVDKKIVPRDCGCKPCICTGGGGSGGGGSGGGGSGGGGSPIEKTISKTKGRPKAPQVYTIPPPKEQMAKDKVSLTCMITDFFPEDITVEWQWNGQPAENYKNTQPIMDTDGSYFVYSKLNVQKSNWEAGNTFTCSVLHEGLHNHHTEKSLSHSPGK

SEQ ID NO: 31 - protein, 362 aa, Artificial Sequence
  delta 231-335
EVHLQQSGPELVKPGASVKMSCKTSGYTFTEYTIHWMKQSHGKSLEWIGGIFPNNGDTTYNQKFKVRATLTVGRSSSTAYMDLRSLTSEDSAVYYCVRNYGSSYGYFDVWGAGTTVTVSSAKTTPPSVYPLAPGSAAQTNSMVTLGCLVKGYFPEPVTVTWNSGSLSSGVHTFPAVLQSDLYTLSSSVTVPSSTWPSETVTCNVAHPASSTKVDKKIVPRDCGCKPCICTGGGGSGGGGSGGGGSGGGGSISKTKGRPKAPQVYTIPPPKEQMAKDKVSLTCMITDFFPEDITVEWQWNGQPAENYKNTQPIMDTDGSYFVYSKLNVQKSNWEAGNTFTCSVLHEGLHNHHTEKSLSHSPGK

SEQ ID NO: 32 - protein, 356 aa, Artificial Sequence
  delta 231-335
QVQLQQSGAELARPGASVKLSCKASGYTFTSQWLQWVKQRPGQGLEWIGAIYPGDGDTRYTQKFKGKATLTADKSSSTAYMQLTNLAPEDSAVYYCARSSMDYWGQGTSVTVSSAKTTPPSVYPLAPGSAAQTNSMVTLGCLVKGYFPEPVTVTWNSGSLSSGVHTFPAVLQSDLYTLSSSVTVPSSTWPSETVTCNVAHPASSTKVDKKIVPRDCGCKPCICTGGGGSGGGGSGGGGSGGGGSISKTKGRPKAPQVYTIPPPKEQMAKDKVSLTCMITDFFPEDITVEWQWNGQPAENYKNTQPIMDTDGSYFVYSKLNVQKSNWEAGNTFTCSVLHEGLHNHHTEKSLSHSPGK

SEQ ID NO: 33 - protein, 352 aa, Artificial Sequence
  delta 231-345
EVHLQQSGPELVKPGASVKMSCKTSGYTFTEYTIHWMKQSHGKSLEWIGGIFPNNGDTTYNQKFKVRATLTVGRSSSTAYMDLRSLTSEDSAVYYCVRNYGSSYGYFDVWGAGTTVTVSSAKTTPPSVYPLAPGSAAQTNSMVTLGCLVKGYFPEPVTVTWNSGSLSSGVHTFPAVLQSDLYTLSSSVTVPSSTWPSETVTCNVAHPASSTKVDKKIVPRDCGCKPCICTGGGGSGGGGSGGGGSGGGGSPQVYTIPPPKEQMAKDKVSLTCMITDFFPEDITVEWQWNGQPAENYKNTQPIMDTDGSYFVYSKLNVQKSNWEAGNTFTCSVLHEGLHNHHTEKSLSHSPGK

SEQ ID NO: 34 - protein, 346 aa, Artificial Sequence
  delta 231-345
QVQLQQSGAELARPGASVKLSCKASGYTFTSQWLQWVKQRPGQGLEWIGAIYPGDGDTRYTQKFKGKATLTADKSSSTAYMQLTNLAPEDSAVYYCARSSMDYWGQGTSVTVSSAKTTPPSVYPLAPGSAAQTNSMVTLGCLVKGYFPEPVTVTWNSGSLSSGVHTFPAVLQSDLYTLSSSVTVPSSTWPSETVTCNVAHPASSTKVDKKIVPRDCGCKPCICTGGGGSGGGGSGGGGSGGGGSPQVYTIPPPKEQMAKDKVSLTCMITDFFPEDITVEWQWNGQPAENYKNTQPIMDTDGSYFVYSKLNVQKSNWEAGNTFTCSVLHEGLHNHHTEKSLSHSPGK

SEQ ID NO: 35 - protein, 347 aa, Artificial Sequence
  delta 231-350
EVHLQQSGPELVKPGASVKMSCKTSGYTFTEYTIHWMKQSHGKSLEWIGGIFPNNGDTTYNQKFKVRATLTVGRSSSTAYMDLRSLTSEDSAVYYCVRNYGSSYGYFDVWGAGTTVTVSSAKTTPPSVYPLAPGSAAQTNSMVTLGCLVKGYFPEPVTVTWNSGSLSSGVHTFPAVLQSDLYTLSSSVTVPSSTWPSETVTCNVAHPASSTKVDKKIVPRDCGCKPCICTGGGGSGGGGSGGGGSGGGGSIPPPKEQMAKDKVSLTCMITDFFPEDITVEWQWNGQPAENYKNTQPIMDTDGSYFVYSKLNVQKSNWEAGNTFTCSVLHEGLHNHHTEKSLSHSPGK

SEQ ID NO: 36 - protein, 341 aa, Artificial Sequence
  delta 231-350
QVQLQQSGAELARPGASVKLSCKASGYTFTSQWLQWVKQRPGQGLEWIGAIYPGDGDTRYTQKFKGKATLTADKSSSTAYMQLTNLAPEDSAVYYCARSSMDYWGQGTSVTVSSAKTTPPSVYPLAPGSAAQTNSMVTLGCLVKGYFPEPVTVTWNSGSLSSGVHTFPAVLQSDLYTLSSSVTVPSSTWPSETVTCNVAHPASSTKVDKKIVPRDCGCKPCICTGGGGSGGGGSGGGGSGGGGSIPPPKEQMAKDKVSLTCMITDFFPEDITVEWQWNGQPAENYKNTQPIMDTDGSYFVYSKLNVQKSNWEAGNTFTCSVLHEGLHNHHTEKSLSHSPGK